European Patent Application EP 4 506 016 A2, published February 12, 2025. Title: Pharmaceutical composition comprising anti-human TSLP Receptor antibody. Applicant: Upstream Bio, Inc. Application EP. The sequence listing filed with the application follows.

SEQUENCE LISTING (4 sequences)

SEQ ID NO: 1 - protein, 448 aa, synthetic construct
  REGION 1..448: note = H-chain of anti-human TSLP Receptor antibody
EVQLLESGGGLVQPGGSLRLSCAASGFTFRSSAMHWVRQAPGKGLKWVSSVSGSGAGTYYADSVKGRFTISRDNPKNTLYLQMNSLRAEDTAVYYCVKEGGSRGFDYWGQGTLVTVSSASTKGPSVFPLAPSSKSTSGGTAALGCLVKDYFPEPVTVSWNSGALTSGVHTFPAVLQSSGLYSLSSVVTVPSSSLGTQTYICNVNHKPSNTKVDKKVEPKSCDKTHTCPPCPAPELLGGPSVFLFPPKPKDTLMISRTPEVTCVVVDVSHEDPEVKFNWYVDGVEVHNAKTKPREEQYNSTYRVVSVLTVLHQDWLNGKEYKCKVSNKALPAPIEKTISKAKGQPREPQVYTLPPSRDELTKNQVSLTCLVKGFYPSDIAVEWESNGQPENNYKTTPPVLDSDGSFFLYSKLTVDKSRWQQGNVFSCSVMHEALHNHYTQKSLSLSPGK

SEQ ID NO: 2 - DNA, 1347 bp, synthetic construct
  misc_feature 1..1347: note = H-chain gene of anti-human TSLP Receptor antibody
  source 1..1347: mol_type = other DNA
gaggtgcagctgttggagtctgggggaggcttggtacagccgggggggtccctgagactctcctgtgcagcctctggattcacctttcgcagctctgccatgcattgggtccgccaggctccagggaagggactgaaatgggtctcaagtgttagtggcagtggtgctggaacatactacgcagactccgtgaagggccggttcaccatctccagagacaatcccaagaatacactgtatctgcaaatgaacagtctgagagccgaggacacggccgtatattattgtgtgaaagaagggggcagccggggttttgactactggggccagggaaccctggtcaccgtctcctcagcctccaccaagggcccatcggtcttccccctggcaccctcctccaagagcacctctgggggcacagcggccctgggctgcctggtcaaggactacttccccgaaccggtgacggtgtcgtggaactcaggcgccctgaccagcggcgtgcacaccttcccggctgtcctacagtcctcaggactctactcccttagtagcgtggtgaccgtgccctccagcagcttgggcacccagacctacatctgcaacgtgaatcacaagcccagcaacaccaaggtggacaagaaagttgagcccaaatcttgtgacaaaactcacacatgcccaccgtgcccagcacctgaactcctggggggaccgtcagtcttcctcttccccccaaaacccaaggacaccctcatgatctcccggacccctgaggtcacatgcgtggtggtggacgtgagccacgaagaccctgaggtcaagttcaactggtacgtggacggcgtggaggtgcataatgccaagacaaagccgcgggaggagcagtacaacagcacgtaccgtgtggtcagcgtcctcaccgtcctgcaccaggactggctgaatggcaaggagtacaagtgcaaggtctccaacaaagccctcccagcccccatcgagaaaaccatctccaaagccaaagggcagccccgagaaccacaggtgtacaccctgcccccatcccgggatgagctgaccaagaaccaggtcagcctgacctgcctggtcaaaggcttctatcccagcgacatcgccgtggagtgggagagcaatgggcagccggagaacaactacaagaccacgcctcccgtgctggactccgacggctccttcttcctctacagcaagctcaccgtggacaagagcaggtggcagcaggggaacgtcttctcatgctccgtgatgcatgaggctctgcacaaccactacacgcagaagagcctctccctgtctccgggtaaatga

SEQ ID NO: 3 - protein, 214 aa, synthetic construct
  REGION 1..214: note = L-chain of anti-human TSLP Receptor antibody
DIQMTQSPSSLSASVGDRVTITCRASQDISNYLAWFQQKPGKAPKSLIYTASSLQSGVPSKFSGSGSGTDFTLTISSLQPEDFATYYCQQYNLYPPTFGQGTKVEIKRTVAAPSVFIFPPSDEQLKSGTASVVCLLNNFYPREAKVQWKVDNALQSGNSQESVTEQDSKDSTYSLSSTLTLSKADYEKHKVYACEVTHQGLSSPVTKSFNRGEC

SEQ ID NO: 4 - DNA, 645 bp, synthetic construct
  misc_feature 1..645: note = L-chain gene of anti-human TSLP Receptor antibody
  source 1..645: mol_type = other DNA
gacatccagatgacccagtctccatcctcactgtctgcatctgtaggagacagagtcaccatcacttgtcgggcgagtcaggacattagcaattatttagcctggtttcagcagaaaccagggaaagcccctaagtccctgatctatactgcatccagtttgcaaagtggggtcccatcaaagttcagcggcagtggatctgggacagatttcactctcaccatcagcagcctgcagcctgaagattttgcaacttattactgccaacagtataatctttatcctccgacgttcggccaagggaccaaggtggaaatcaaacggactgtggctgcaccatctgtcttcatcttcccgccatctgatgagcagttgaaatctggaactgcctctgttgtgtgcctgctgaataacttctatcccagagaggccaaagtacagtggaaggtggataacgccctccaatcgggtaactcccaggagagtgtcacagagcaggacagcaaggacagcacctacagcctcagcagcaccctgacgctgagcaaagcagactacgagaaacacaaagtctacgcctgcgaagtcacccatcagggcctgagctcgcccgtcacaaagagcttcaacaggggagagtgttag